European Patent Specification EP 2 885 408 B1, published January 25, 2023. Title: DIGITAL BIOLOGICAL CONVERTER. Applicant: SYNTHETIC GENOMICS, INC. VENTER, J. Craig GIBSON, Daniel G. GILL, John  E. The sequence listing filed with the application follows.

SEQUENCE LISTING (6 sequences)

SEQ ID NO: 1 - DNA, 1400 bp, phi X virus
gagttttatcgcttccatgacgcagaagttaacactttcggatatttctgatgagtcgaaaaattatcttgataaagcaggaattactactgcttgtttacgaattaaatcgaagtggactgctggcggaaaatgagaaaattcgacctatccttgcgcagctcgagaagctcttactttgcgacctttcgccatcaactaacgattctgtcaaaaactgacgcgttggatgaggagaagtggcttaatatgcttggcacgttcgtcaaggactggtttagatatgagtcacattttgttcatggtagagattctcttgttgacattttaaaagagcgtggattactatctgagtccgatgctgttcaaccactaataggtaagaaatcatgagtcaagttactgaacaatccgtacgtttccagaccgctttggcctctattaagctcattcaggcttctgccgttttggatttaaccgaagatgatttcgattttctgacgagtaacaaagtttggattgctactgaccgctctcgtgctcgtcgctgcgttgaggcttgcgtttatggtacgctggactttgtgggataccctcgctttcctgctcctgttgagtttattgctgccgtcattgcttattatgttcatcccgtcaacattcaaacggcctgtctcatcatggaaggcgctgaatttacggaaaacattattaatggcgtcgagcgtccggttaaagccgctgaattgttcgcgtttaccttgcgtgtacgcgcaggaaacactgacgttcttactgacgcagaagaaaacgtgcgtcaaaaattacgtgcggaaggagtgatgtaatgtctaaaggtaaaaaacgttctggcgctcgccctggtcgtccgcagccgttgcgaggtactaaaggcaagcgtaaaggcgctcgtctttggtatgtaggtggtcaacaattttaattgcaggggcttcggccccttacttgaggataaattatgtctaatattcaaactggcgccgagcgtatgccgcatgacctttcccatcttggcttccttgctggtcagattggtcgtcttattaccatttcaactactccggttatcgctggcgactccttcgagatggacgccgttggcgctctccgtctttctccattgcgtcgtggccttgctattgactctactgtagacatttttactttttatgtccctcatcgtcacgtttatggtgaacagtggattaagttcatgaaggatggtgttaatgccactcctctcccgactgttaacactactggttatattgaccatgccgcttttcttggcacgattaaccctgataccaataaaatccctaagcatttgtttcagggttatttgaatatctataaca

SEQ ID NO: 2 - DNA, 1400 bp, phi X virus
cctaagcatttgtttcagggttatttgaatatctataacaactattttaaagcgccgtggatgcctgaccgtaccgaggctaaccctaatgagcttaatcaagatgatgctcgttatggtttccgttgctgccatctcaaaaacatttggactgctccgcttcctcctgagactgagctttctcgccaaatgacgacttctaccacatctattgacattatgggtctgcaagctgcttatgctaatttgcatactgaccaagaacgtgattacttcatgcagcgttaccatgatgttatttcttcatttggaggtaaaacctcttatgacgctgacaaccgtcctttacttgtcatgcgctctaatctctgggcatctggctatgatgttgatggaactgaccaaacgtcgttaggccagttttctggtcgtgttcaacagacctataaacattctgtgccgcgtttctttgttcctgagcatggcactatgtttactcttgcgcttgttcgttttccgcctactgcgactaaagagattcagtaccttaacgctaaaggtgctttgacttataccgatattgctggcgaccctgttttgtatggcaacttgccgccgcgtgaaatttctatgaaggatgttttccgttctggtgattcgtctaagaagtttaagattgctgagggtcagtggtatcgttatgcgccttcgtatgtttctcctgcttatcaccttcttgaaggcttcccattcattcaggaaccgccttctggtgatttgcaagaacgcgtacttattcgccaccatgattatgaccagtgtttccagtccgttcagttgttgcagtggaatagtcaggttaaatttaatgtgaccgtttatcgcaatctgccgaccactcgcgattcaatcatgacttcgtgataaaagattgagtgtgaggttataacgccgaagcggtaaaaattttaatttttgccgctgaggggttgaccaagcgaagcgcggtaggttttctgcttaggagtttaatcatgtttcagacttttatttctcgccataattcaaactttttttctgataagctggttctcacttctgttactccagcttcttcggcacctgttttacagacacctaaagctacatcgtcaacgttatattttgatagtttgacggttaatgctggtaatggtggttttcttcattgcattcagatggatacatctgtcaacgccgctaatcaggttgtttctgttggtgctgatattgcttttgatgccgaccctaaattttttgcctgtttggttcgctttgagtcttcttcggttccgactaccctcccgactgcctatgatgtttatcctttgaatggtcgccatgatggtggttattatacc

SEQ ID NO: 3 - DNA, 1400 bp, phi X virus
ttatcctttgaatggtcgccatgatggtggttattataccgtcaaggactgtgtgactattgacgtccttccccgtacgccgggcaataacgtttatgttggtttcatggtttggtctaactttaccgctactaaatgccgcggattggtttcgctgaatcaggttattaaagagattatttgtctccagccacttaagtgaggtgatttatgtttggtgctattgctggcggtattgcttctgctcttgctggtggcgccatgtctaaattgtttggaggcggtcaaaaagccgcctccggtggcattcaaggtgatgtgcttgctaccgataacaatactgtaggcatgggtgatgctggtattaaatctgccattcaaggctctaatgttcctaaccctgatgaggccgcccctagttttgtttctggtgctatggctaaagctggtaaaggacttcttgaaggtacgttgcaggctggcacttctgccgtttctgataagttgcttgatttggttggacttggtggcaagtctgccgctgataaaggaaaggatactcgtgattatcttgctgctgcatttcctgagcttaatgcttgggagcgtgctggtgctgatgcttcctctgctggtatggttgacgccggatttgagaatcaaaaagagcttactaaaatgcaactggacaatcagaaagagattgccgagatgcaaaatgagactcaaaaagagattgctggcattcagtcggcgacttcacgccagaatacgaaagaccaggtatatgcacaaaatgagatgcttgcttatcaacagaaggagtctactgctcgcgttgcgtctattatggaaaacaccaatctttccaagcaacagcaggtttccgagattatgcgccaaatgcttactcaagctcaaacggctggtcagtattttaccaatgaccaaatcaaagaaatgactcgcaaggttagtgctgaggttgacttagttcatcagcaaacgcagaatcagcggtatggctcttctcatattggcgctactgcaaaggatatttctaatgtcgtcactgatgctgcttctggtgtggttgatatttttcatggtattgataaagctgttgccgatacttggaacaatttctggaaagacggtaaagctgatggtattggctctaatttgtctaggaaataaccgtcaggattgacaccctcccaattgtatgttttcatgcctccaaatcttggaggcttttttatggttcgttcttattacccttctgaatgtcacgctgattattttgactttgagcgtatcgaggctcttaaacctgctattgaggcttgtggcatttctactctttctcaatccccaatgcttggcttccataagcagat

SEQ ID NO: 4 - DNA, 1346 bp, phi X virus
ctctttctcaatccccaatgcttggcttccataagcagatggataaccgcatcaagctcttggaagagattctgtcttttcgtatgcagggcgttgagttcgataatggtgatatgtatgttgacggccataaggctgcttctgacgttcgtgatgagtttgtatctgttactgagaagttaatggatgaattggcacaatgctacaatgtgctcccccaacttgatattaataacactatagaccaccgccccgaaggggacgaaaaatggtttttagagaacgagaagacggttacgcagttttgccgcaagctggctgctgaacgccctcttaaggatattcgcgatgagtataattaccccaaaaagaaaggtattaaggatgagtgttcaagattgctggaggcctccactatgaaatcgcgtagaggctttgctattcagcgtttgatgaatgcaatgcgacaggctcatgctgatggttggtttatcgtttttgacactctcacgttggctgacgaccgattagaggcgttttatgataatcccaatgctttgcgtgactattttcgtgatattggtcgtatggttcttgctgccgagggtcgcaaggctaatgattcacacgccgactgctatcagtatttttgtgtgcctgagtatggtacagctaatggccgtcttcatttccatgcggtgcactttatgcggacacttcctacaggtagcgttgaccctaattttggtcgtcgggtacgcaatcgccgccagttaaatagcttgcaaaatacgtggccttatggttacagtatgcccatcgcagttcgctacacgcaggacgctttttcacgttctggttggttgtggcctgttgatgctaaaggtgagccgcttaaagctaccagttatatggctgttggtttctatgtggctaaatacgttaacaaaaagtcagatatggaccttgctgctaaaggtctaggagctaaagaatggaacaactcactaaaaaccaagctgtcgctacttcccaagaagctgttcagaatcagaatgagccgcaacttcgggatgaaaatgctcacaatgacaaatctgtccacggagtgcttaatccaacttaccaagctgggttacgacgcgacgccgttcaaccagatattgaagcagaacgcaaaaagagagatgagattgaggctgggaaaagttactgtagccgacgttttggcggcgcaacctgtgacgacaaatctgctcaaatttatgcgcgcttcgataaaaatgattggcgtatccaacctgcagagttttatcgcttccatgacgcagaagttaacactttcg

SEQ ID NO: 5 - DNA, 5386 bp, phi X virus
gagttttatcgcttccatgacgcagaagttaacactttcggatatttctgatgagtcgaaaaattatcttgataaagcaggaattactactgcttgtttacgaattaaatcgaagtggactgctggcggaaaatgagaaaattcgacctatccttgcgcagctcgagaagctcttactttgcgacctttcgccatcaactaacgattctgtcaaaaactgacgcgttggatgaggagaagtggcttaatatgcttggcacgttcgtcaaggactggtttagatatgagtcacattttgttcatggtagagattctcttgttgacattttaaaagagcgtggattactatctgagtccgatgctgttcaaccactaataggtaagaaatcatgagtcaagttactgaacaatccgtacgtttccagaccgctttggcctctattaagctcattcaggcttctgccgttttggatttaaccgaagatgatttcgattttctgacgagtaacaaagtttggattgctactgaccgctctcgtgctcgtcgctgcgttgaggcttgcgtttatggtacgctggactttgtgggataccctcgctttcctgctcctgttgagtttattgctgccgtcattgcttattatgttcatcccgtcaacattcaaacggcctgtctcatcatggaaggcgctgaatttacggaaaacattattaatggcgtcgagcgtccggttaaagccgctgaattgttcgcgtttaccttgcgtgtacgcgcaggaaacactgacgttcttactgacgcagaagaaaacgtgcgtcaaaaattacgtgcggaaggagtgatgtaatgtctaaaggtaaaaaacgttctggcgctcgccctggtcgtccgcagccgttgcgaggtactaaaggcaagcgtaaaggcgctcgtctttggtatgtaggtggtcaacaattttaattgcaggggcttcggccccttacttgaggataaattatgtctaatattcaaactggcgccgagcgtatgccgcatgacctttcccatcttggcttccttgctggtcagattggtcgtcttattaccatttcaactactccggttatcgctggcgactccttcgagatggacgccgttggcgctctccgtctttctccattgcgtcgtggccttgctattgactctactgtagacatttttactttttatgtccctcatcgtcacgtttatggtgaacagtggattaagttcatgaaggatggtgttaatgccactcctctcccgactgttaacactactggttatattgaccatgccgcttttcttggcacgattaaccctgataccaataaaatccctaagcatttgtttcagggttatttgaatatctataacaactattttaaagcgccgtggatgcctgaccgtaccgaggctaaccctaatgagcttaatcaagatgatgctcgttatggtttccgttgctgccatctcaaaaacatttggactgctccgcttcctcctgagactgagctttctcgccaaatgacgacttctaccacatctattgacattatgggtctgcaagctgcttatgctaatttgcatactgaccaagaacgtgattacttcatgcagcgttaccatgatgttatttcttcatttggaggtaaaacctcttatgacgctgacaaccgtcctttacttgtcatgcgctctaatctctgggcatctggctatgatgttgatggaactgaccaaacgtcgttaggccagttttctggtcgtgttcaacagacctataaacattctgtgccgcgtttctttgttcctgagcatggcactatgtttactcttgcgcttgttcgttttccgcctactgcgactaaagagattcagtaccttaacgctaaaggtgctttgacttataccgatattgctggcgaccctgttttgtatggcaacttgccgccgcgtgaaatttctatgaaggatgttttccgttctggtgattcgtctaagaagtttaagattgctgagggtcagtggtatcgttatgcgccttcgtatgtttctcctgcttatcaccttcttgaaggcttcccattcattcaggaaccgccttctggtgatttgcaagaacgcgtacttattcgccaccatgattatgaccagtgtttccagtccgttcagttgttgcagtggaatagtcaggttaaatttaatgtgaccgtttatcgcaatctgccgaccactcgcgattcaatcatgacttcgtgataaaagattgagtgtgaggttataacgccgaagcggtaaaaattttaatttttgccgctgaggggttgaccaagcgaagcgcggtaggttttctgcttaggagtttaatcatgtttcagacttttatttctcgccataattcaaactttttttctgataagctggttctcacttctgttactccagcttcttcggcacctgttttacagacacctaaagctacatcgtcaacgttatattttgatagtttgacggttaatgctggtaatggtggttttcttcattgcattcagatggatacatctgtcaacgccgctaatcaggttgtttctgttggtgctgatattgcttttgatgccgaccctaaattttttgcctgtttggttcgctttgagtcttcttcggttccgactaccctcccgactgcctatgatgtttatcctttgaatggtcgccatgatggtggttattataccgtcaaggactgtgtgactattgacgtccttccccgtacgccgggcaataacgtttatgttggtttcatggtttggtctaactttaccgctactaaatgccgcggattggtttcgctgaatcaggttattaaagagattatttgtctccagccacttaagtgaggtgatttatgtttggtgctattgctggcggtattgcttctgctcttgctggtggcgccatgtctaaattgtttggaggcggtcaaaaagccgcctccggtggcattcaaggtgatgtgcttgctaccgataacaatactgtaggcatgggtgatgctggtattaaatctgccattcaaggctctaatgttcctaaccctgatgaggccgcccctagttttgtttctggtgctatggctaaagctggtaaaggacttcttgaaggtacgttgcaggctggcacttctgccgtttctgataagttgcttgatttggttggacttggtggcaagtctgccgctgataaaggaaaggatactcgtgattatcttgctgctgcatttcctgagcttaatgcttgggagcgtgctggtgctgatgcttcctctgctggtatggttgacgccggatttgagaatcaaaaagagcttactaaaatgcaactggacaatcagaaagagattgccgagatgcaaaatgagactcaaaaagagattgctggcattcagtcggcgacttcacgccagaatacgaaagaccaggtatatgcacaaaatgagatgcttgcttatcaacagaaggagtctactgctcgcgttgcgtctattatggaaaacaccaatctttccaagcaacagcaggtttccgagattatgcgccaaatgcttactcaagctcaaacggctggtcagtattttaccaatgaccaaatcaaagaaatgactcgcaaggttagtgctgaggttgacttagttcatcagcaaacgcagaatcagcggtatggctcttctcatattggcgctactgcaaaggatatttctaatgtcgtcactgatgctgcttctggtgtggttgatatttttcatggtattgataaagctgttgccgatacttggaacaatttctggaaagacggtaaagctgatggtattggctctaatttgtctaggaaataaccgtcaggattgacaccctcccaattgtatgttttcatgcctccaaatcttggaggcttttttatggttcgttcttattacccttctgaatgtcacgctgattattttgactttgagcgtatcgaggctcttaaacctgctattgaggcttgtggcatttctactctttctcaatccccaatgcttggcttccataagcagatggataaccgcatcaagctcttggaagagattctgtcttttcgtatgcagggcgttgagttcgataatggtgatatgtatgttgacggccataaggctgcttctgacgttcgtgatgagtttgtatctgttactgagaagttaatggatgaattggcacaatgctacaatgtgctcccccaacttgatattaataacactatagaccaccgccccgaaggggacgaaaaatggtttttagagaacgagaagacggttacgcagttttgccgcaagctggctgctgaacgccctcttaaggatattcgcgatgagtataattaccccaaaaagaaaggtattaaggatgagtgttcaagattgctggaggcctccactatgaaatcgcgtagaggctttgctattcagcgtttgatgaatgcaatgcgacaggctcatgctgatggttggtttatcgtttttgacactctcacgttggctgacgaccgattagaggcgttttatgataatcccaatgctttgcgtgactattttcgtgatattggtcgtatggttcttgctgccgagggtcgcaaggctaatgattcacacgccgactgctatcagtatttttgtgtgcctgagtatggtacagctaatggccgtcttcatttccatgcggtgcactttatgcggacacttcctacaggtagcgttgaccctaattttggtcgtcgggtacgcaatcgccgccagttaaatagcttgcaaaatacgtggccttatggttacagtatgcccatcgcagttcgctacacgcaggacgctttttcacgttctggttggttgtggcctgttgatgctaaaggtgagccgcttaaagctaccagttatatggctgttggtttctatgtggctaaatacgttaacaaaaagtcagatatggaccttgctgctaaaggtctaggagctaaagaatggaacaactcactaaaaaccaagctgtcgctacttcccaagaagctgttcagaatcagaatgagccgcaacttcgggatgaaaatgctcacaatgacaaatctgtccacggagtgcttaatccaacttaccaagctgggttacgacgcgacgccgttcaaccagatattgaagcagaacgcaaaaagagagatgagattgaggctgggaaaagttactgtagccgacgttttggcggcgcaacctgtgacgacaaatctgctcaaatttatgcgcgcttcgataaaaatgattggcgtatccaacctgca

SEQ ID NO: 6 - DNA, 10 bp, phi X virus
acgttgcagc